European Patent Specification EP 3 704 143 B1, published October 18, 2023. Title: Chemo-enzymatic Synthesis of Liraglutide, Semaglutide and GLP-1. Applicant: EnzyPep B.V. The sequence listing filed with the application follows.

SEQUENCE LISTING (14 sequences)

SEQ ID NO: 1 - DNA, 1149 bp, Bacillus amyloliquefaciens
  CDS (322)..(1149)
gtgagaggcaaaaaagtatggatcagtttgctgtttgctttagcgttaatctttacgatggcgttcggcagcacatcctctgcccaggcggcagggaaatcaaacggggaaaagaaatatattgtcgggtttaaacagacaatgagcacgatgagcgccgctaagaagaaagatgtcatttctgaaaaaggcgggaaagtgcaaaagcaattcaaatatgtagacgcagcttcagctacattaaacgaaaaagctgtaaaagaattgaaaaaagacccgagcgtcgcttacgttgaagaagatcacgtagcacatgcgtacgcgcagtccgtgccttacggcgtatcacaaattaaagcccctgctctgcactctcaaggctacactggatcaaatgttaaagtagcggttatcgacagcggtatcgattcttctcatcctgatttaaaggtagcaggcggagccagcatggttccttctgaaacaaatcctttccaagacaacaactctcacggaactcacgttgccggcacagttgcggctcttaataactcaatcggtgtattaggcgttgcgccaagcgcatcactttacgctgtaaaagttctcggtgctgacggttccggccaatacagctggatcattaacggaatcgagtgggcgatcgcaaacaatatggacgttattaacatgagcctcggcggaccttctggttctgctgctttaaaagcggcagttgataaagccgttgcatccggcgtcgtagtcgttgcggcagccggtaacgaaggcacttccggcagctcaagcacagtgggctaccctggtaaatacccttctgtcattgcagtaggcgctgttgacagcagcaaccaaagagcatctttctcaagcgtaggacctgagcttgatgtcatggcacctggcgtatctatccaaagcacgcttcctggaaacaaatacggggcgtacaacggtacgtcaatggcatctccgcacgttgccggagcggctgctttgattctttctaagcacccgaactggacaaacactcaagtccgcagcagtttagaaaacaccactacaaaacttggtgattctttctactatggaaaagggctgatcaacgtacaggcggcagctcagtaa

SEQ ID NO: 2 - protein, 275 aa, Bacillus amyloliquefaciens [sequence omitted]

SEQ ID NO: 3 - protein, 272 aa, Artificial Sequence
  mutant subtilisin B
  MISC_FEATURE (267)..(272): His-tag
AKCVSYGVAQIKAPALHSQGYTGSNVKVAVLDSGIDSSHPDLNVAGGASFVPSETNPFQDNASHGTHVAGTVLAVAPSASLYAVKVLGADGSGQYSWIINGIEWAIANNMDVINMSLGGPSGSAALKAAVDKAVASGVVVVAAAGNNGTSGSSSTVEYPAKYPSVIAVGAVDSSNQRAPWSSVGPELDVMAPGVSICSTLPGGKYGAHDGTCPASNHVAGAAALILSKHPNWTNTQVRSSLENTATKLGDSFYYGKGLINVEAAAQHHHHHH

SEQ ID NO: 4 - protein, 31 aa, Artificial Sequence
  consensus peptide fragment
  VARIANT (2)..(2): may also be an alpha-amino-isobutyric acid unit
  MISC_FEATURE (20)..(20): Lys has a free side-chain epsilon-amino group or a side-chain epsilon-amino group that is protected with a protective group or a side-chain epsilon-amino group that is functionalised with an amino acid or another functional group
  VARIANT (28)..(28): may also be K
HAEGTFTSDVSSYLEGQAAKEFIAWLVRGRG

SEQ ID NO: 5 - protein, 31 aa, Homo sapiens
HAEGTFTSDVSSYLEGQAAKEFIAWLVKGRG

SEQ ID NO: 6 - protein, 31 aa, Homo sapiens; identical to SEQ ID NO: 5
  MOD_RES (20)..(20): Lys is Lys(Pal-gamma-Glu)-
  MOD_RES (20)..(20): Lys is Lys(Pal-gamma-Glu)

SEQ ID NO: 7 - protein, 31 aa, Homo sapiens; identical to SEQ ID NO: 5
  MOD_RES (2)..(2): bAib
  MOD_RES (20)..(20): Lys is Lys(AEEA-AEEA-gamma-Glu-17-carboxyheptadecanoyl)

SEQ ID NO: 8 - protein, 27 aa, Artificial Sequence
  coupling reagent for production of liraglutide
  MOD_RES (20)..(20): Lys is Lys(Pal-Glu-OX) in which X is H or protective group
TFTSDVSSYLEGQAAKEFIAWLVRGRG

SEQ ID NO: 9 - protein, 14 aa, Artificial Sequence
  13-mer C-terminal ester for coupling
  MOD_RES (14)..(14): is OCam-Leu
HAEGTFTSDVSSYL

SEQ ID NO: 10 - protein, 18 aa, Artificial Sequence
  18-mer coupling peptide
LEGQAAKEFIAWLVRGRG

SEQ ID NO: 11 - protein, 11 aa, Artificial Sequence
  11-mer coupling peptide
  VARIANT (2)..(2): may also be an alpha-amino-isobutyric acid unit
  MOD_RES (11)..(11): thioester
HAEGTFTSDVS

SEQ ID NO: 12 - protein, 20 aa, Artificial Sequence
  20-mer coupling peptide
  MISC_FEATURE (9)..(9): Lys has a free side-chain epsilon-amino group or a side-chain epsilon-amino group that is protected with a protective group or a side-chain epsilon-amino group that is functionalised with an amino acid or another functional group
  MOD_RES (17)..(17): May also be Lys
SYLEGQAAKEFIAWLVRGRG

SEQ ID NO: 13 - protein, 20 aa, Artificial Sequence
  20-mer coupling peptide
  MOD_RES (9)..(9): Lys(Pal-gamma-Glu-OH)
  MOD_RES (9)..(9): Lys(Pal-gamma-Glu-OH) or Lys(gamma-Glu-OH)
SYLEGQAAKEFIAWLVRGRG

SEQ ID NO: 14 - protein, 272 aa, artificial sequence
  mutant subtilisin B
  MISC_FEATURE (267)..(272): His-tag
AKCVSYGVAQIKAPALHSQGYTGSNVKVAVLDSGIDSSHPDLNVAGGASFVPSETNPFQDNNSHGTHVAGTVLAVAPSASLYAVKVLGADGSGQYSWIINGIEWAIANNMDVINMSLGGPSGSAALKAAVDKAVASGVVVVAAAGNSGTSGSSSTVSYPAKYPSVIAVGAVDSSNQRAPFSSVGPELDVMAPGVSICSTLPGGKYGAHSGTCPASNHVAGAAALILSKHPNWTNTQVRSSLENTATKLGDSFYYGKGLINVEAAAQHHHHHH